European Patent Application EP 4 613 771 A1, published September 10, 2025. Title: Chimeric antigen receptor with elevated affinity for mesothelin and uses thereof. Applicant: Cellengene Inc. The sequence listing filed with the application follows.

SEQUENCE LISTING (60 sequences)

SEQ ID NO: 1 - protein, 243 aa, synthetic construct
EVQLVESGGGLVQPGGSLRLSCAASGFTFSDYGMHWVRQAPGKGLEWVSSIYGSGGHTGYADSVKGRFTISRDNSKNTLYLQMNSLRAEDTAVYYCAKQHAYRYSYAFDVWGQGTLVTVSSGGGGSGGGGSGGGGSDIQMTQSPSSLSASVGDRVTITCRASQSISNWLNWYQQKPGKAPKLLIYATSSLQSGVPSRFSGSGSGTDFTLTISSLQPEDFATYYCQQSYSFPFTFGQGTKVEIK

SEQ ID NO: 2 - protein, 243 aa, synthetic construct
EVQLVESGGGLVQPGGSLRLSCAASGFTFSLYGMHWVRQAPGKGLEWVSSIYGSGGHTGYADSVKGRFTISRDNSKNTLYLQMNSLRAEDTAVYYCAKQHAYRYSYAFDVWGQGTLVTVSSGGGGSGGGGSGGGGSDIQMTQSPSSLSASVGDRVTITCRASQSISNWLNWYQQKPGKAPKLLIYATSSLQSGVPSRFSGSGSGTDFTLTISSLQPEDFATYYCQQSYSFPFTFGQGTKVEIK

SEQ ID NO: 3 - protein, 243 aa, synthetic construct
EVQLVESGGGLVQPGGSLRLSCAASGFTFSDYGMHWVRQAPGKGLEWVSSIYGSGGHTGYADSVKGRFTISRDNSKNTLYLQMNSLRAEDTAVYYCAKQHAYRYSYAFDVWGQGTLVTVSSGGGGSGGGGSGGGGSDIQMTQSPSSLSASVGDRVTITCRASQSISNWLNWYQQKPGKAPKLLIYATSSLQRGVPSRFSGSGSGTDFTLTISSLQPEDFATYYCQQSYSFPFTFGQGTKVEIK

SEQ ID NO: 4 - protein, 243 aa, synthetic construct
EVQLVESGGGLVQPGGSLRLSCAASGFTFSLYGMHWVRQAPGKGLEWVSSIYGSGGHTGYADSVKGRFTISRDNSKNTLYLQMNSLRAEDTAVYYCAKQHAYRYSYAFDVWGQGTLVTVSSGGGGSGGGGSGGGGSDIQMTQSPSSLSASVGDRVTITCRASQSISNWLNWYQQKPGKAPKLLIYATSSLQRGVPSRFSGSGSGTDFTLTISSLQPEDFATYYCQQSYSFPFTFGQGTKVEIK

SEQ ID NO: 5 - DNA, 23 bp, synthetic construct
  source 1..23: mol_type = other DNA
aaatatggtatgcactgggttcg

SEQ ID NO: 6 - DNA, 30 bp, synthetic construct
  source 1..30: mol_type = other DNA
ataccatatttagagaaagtaaaacccgag

SEQ ID NO: 7 - DNA, 27 bp, synthetic construct
  source 1..27: mol_type = other DNA
ctcttggtatggtatgcactgggttcg

SEQ ID NO: 8 - DNA, 30 bp, synthetic construct
  source 1..30: mol_type = other DNA
ataccataccaagagaaagtaaaacccgag

SEQ ID NO: 9 - DNA, 27 bp, synthetic construct
  source 1..27: mol_type = other DNA
ctctctgtatggtatgcactgggttcg

SEQ ID NO: 10 - DNA, 30 bp, synthetic construct
  source 1..30: mol_type = other DNA
ataccatacagagagaaagtaaaacccgag

SEQ ID NO: 11 - DNA, 27 bp, synthetic construct
  source 1..27: mol_type = other DNA
ctctcgttatggtatgcactgggttcg

SEQ ID NO: 12 - DNA, 30 bp, synthetic construct
  source 1..30: mol_type = other DNA
ataccataacgagagaaagtaaaacccgag

SEQ ID NO: 13 - DNA, 22 bp, synthetic construct
  source 1..22: mol_type = other DNA
gcagtttggtgtaccgtcccgt

SEQ ID NO: 14 - DNA, 25 bp, synthetic construct
  source 1..25: mol_type = other DNA
ggtacaccaaactgcagagaggaag

SEQ ID NO: 15 - DNA, 22 bp, synthetic construct
  source 1..22: mol_type = other DNA
gcagcgtggtgtaccgtcccgt

SEQ ID NO: 16 - DNA, 25 bp, synthetic construct
  source 1..25: mol_type = other DNA
ggtacaccacgctgcagagaggaag

SEQ ID NO: 17 - DNA, 23 bp, synthetic construct
  source 1..23: mol_type = other DNA
cgctcttttccgtttacgttcgg

SEQ ID NO: 18 - DNA, 29 bp, synthetic construct
  source 1..29: mol_type = other DNA
aaacggaaaagagcgagattgctgacaat

SEQ ID NO: 19 - protein, 5 aa, synthetic construct
DYGMH

SEQ ID NO: 20 - protein, 17 aa, synthetic construct
SIYGSGGHTGYADSVKG

SEQ ID NO: 21 - protein, 12 aa, synthetic construct
QHAYRYSYAFDV

SEQ ID NO: 22 - protein, 11 aa, synthetic construct
RASQSISNWLN

SEQ ID NO: 23 - protein, 7 aa, synthetic construct
ATSSLQS

SEQ ID NO: 24 - protein, 9 aa, synthetic construct
QQSYSFPFT

SEQ ID NO: 25 - protein, 121 aa, synthetic construct
EVQLVESGGGLVQPGGSLRLSCAASGFTFSDYGMHWVRQAPGKGLEWVSSIYGSGGHTGYADSVKGRFTISRDNSKNTLYLQMNSLRAEDTAVYYCAKQHAYRYSYAFDVWGQGTLVTVSS

SEQ ID NO: 26 - protein, 107 aa, synthetic construct
DIQMTQSPSSLSASVGDRVTITCRASQSISNWLNWYQQKPGKAPKLLIYATSSLQSGVPSRFSGSGSGTDFTLTISSLQPEDFATYYCQQSYSFPFTFGQGTKVEIK

SEQ ID NO: 27 - protein, 5 aa, synthetic construct
LYGMH

SEQ ID NO: 28 - protein, 17 aa, synthetic construct
SIYGSGGHTGYADSVKG

SEQ ID NO: 29 - protein, 12 aa, synthetic construct
QHAYRYSYAFDV

SEQ ID NO: 30 - protein, 11 aa, synthetic construct
RASQSISNWLN

SEQ ID NO: 31 - protein, 7 aa, synthetic construct
ATSSLQS

SEQ ID NO: 32 - protein, 9 aa, synthetic construct
QQSYSFPFT

SEQ ID NO: 33 - protein, 121 aa, synthetic construct
EVQLVESGGGLVQPGGSLRLSCAASGFTFSLYGMHWVRQAPGKGLEWVSSIYGSGGHTGYADSVKGRFTISRDNSKNTLYLQMNSLRAEDTAVYYCAKQHAYRYSYAFDVWGQGTLVTVSS

SEQ ID NO: 34 - protein, 107 aa, synthetic construct; identical to SEQ ID NO: 26

SEQ ID NO: 35 - protein, 5 aa, synthetic construct
DYGMH

SEQ ID NO: 36 - protein, 17 aa, synthetic construct
SIYGSGGHTGYADSVKG

SEQ ID NO: 37 - protein, 12 aa, synthetic construct
QHAYRYSYAFDV

SEQ ID NO: 38 - protein, 11 aa, synthetic construct
RASQSISNWLN

SEQ ID NO: 39 - protein, 7 aa, synthetic construct
ATSSLQR

SEQ ID NO: 40 - protein, 9 aa, synthetic construct
QQSYSFPFT

SEQ ID NO: 41 - protein, 121 aa, synthetic construct; identical to SEQ ID NO: 25

SEQ ID NO: 42 - protein, 107 aa, synthetic construct
DIQMTQSPSSLSASVGDRVTITCRASQSISNWLNWYQQKPGKAPKLLIYATSSLQRGVPSRFSGSGSGTDFTLTISSLQPEDFATYYCQQSYSFPFTFGQGTKVEIK

SEQ ID NO: 43 - protein, 5 aa, synthetic construct
LYGMH

SEQ ID NO: 44 - protein, 17 aa, synthetic construct
SIYGSGGHTGYADSVKG

SEQ ID NO: 45 - protein, 12 aa, synthetic construct
QHAYRYSYAFDV

SEQ ID NO: 46 - protein, 11 aa, synthetic construct
RASQSISNWLN

SEQ ID NO: 47 - protein, 7 aa, synthetic construct
ATSSLQR

SEQ ID NO: 48 - protein, 9 aa, synthetic construct
QQSYSFPFT

SEQ ID NO: 49 - protein, 121 aa, synthetic construct; identical to SEQ ID NO: 33

SEQ ID NO: 50 - protein, 107 aa, synthetic construct; identical to SEQ ID NO: 42

SEQ ID NO: 51 - DNA, 63 bp, synthetic construct
  source 1..63: mol_type = other DNA
atggccttaccagtgaccgccttgctcctgccgctggccttgctgctccacgccgccaggccg

SEQ ID NO: 52 - DNA, 729 bp, synthetic construct
  source 1..729: mol_type = other DNA
gaagtacagttggtcgaaagtggcggtggcctcgtgcaaccgggtggttcactgcgtctgagctgcgccgcctcgggttttactttctctgattatggtatgcactgggttcgtcaggcgccgggcaagggtctcgaatgggtttcatctatctacggttctggtggtcacactggttatgccgattcagtgaagggtcgctttaccatttcccgtgacaactctaagaatactctgtatctgcagatgaactcgctgcgtgccgaagacacggccgtctattattgcgccaaacagcatgcataccgttactcttacgcattcgatgtttggggtcagggcactttagtgaccgtctcatcgggtggaggcggttcaggcggaggtggatccggcggtggcggatcggacattcaaatgacgcagagtccctcctcactgagtgctagcgtgggcgatcgtgtgacaattacttgtcgcgctagccagtctatctctaattggctgaactggtatcagcagaaaccgggcaaggcgccaaaattgctgatttacgcaacttcctctctgcagtctggtgtaccgtcccgtttctctggcagcggttctggtacggattttaccctgaccatctcaagcctccagcctgaagattttgccacctattattgtcagcaatcttactcttttccgtttacgttcgggcagggaactaaagtggaaattaaa

SEQ ID NO: 53 - DNA, 729 bp, synthetic construct
  source 1..729: mol_type = other DNA
gaagtacagttggtcgaaagtggcggtggcctcgtgcaaccgggtggttcactgcgtctgagctgcgccgcctcgggttttactttctctctttatggtatgcactgggttcgtcaggcgccgggcaagggtctcgaatgggtttcatctatctacggttctggtggtcacactggttatgccgattcagtgaagggtcgctttaccatttcccgtgacaactctaagaatactctgtatctgcagatgaactcgctgcgtgccgaagacacggccgtctattattgcgccaaacagcatgcataccgttactcttacgcattcgatgtttggggtcagggcactttagtgaccgtctcatcgggtggaggcggttcaggcggaggtggatccggcggtggcggatcggacattcaaatgacgcagagtccctcctcactgagtgctagcgtgggcgatcgtgtgacaattacttgtcgcgctagccagtctatctctaattggctgaactggtatcagcagaaaccgggcaaggcgccaaaattgctgatttacgcaacttcctctctgcagtctggtgtaccgtcccgtttctctggcagcggttctggtacggattttaccctgaccatctcaagcctccagcctgaagattttgccacctattattgtcagcaatcttactcttttccgtttacgttcgggcagggaactaaagtggaaattaaa

SEQ ID NO: 54 - DNA, 729 bp, synthetic construct
  source 1..729: mol_type = other DNA
gaagtacagttggtcgaaagtggcggtggcctcgtgcaaccgggtggttcactgcgtctgagctgcgccgcctcgggttttactttctctgattatggtatgcactgggttcgtcaggcgccgggcaagggtctcgaatgggtttcatctatctacggttctggtggtcacactggttatgccgattcagtgaagggtcgctttaccatttcccgtgacaactctaagaatactctgtatctgcagatgaactcgctgcgtgccgaagacacggccgtctattattgcgccaaacagcatgcataccgttactcttacgcattcgatgtttggggtcagggcactttagtgaccgtctcatcgggtggaggcggttcaggcggaggtggatccggcggtggcggatcggacattcaaatgacgcagagtccctcctcactgagtgctagcgtgggcgatcgtgtgacaattacttgtcgcgctagccagtctatctctaattggctgaactggtatcagcagaaaccgggcaaggcgccaaaattgctgatttacgcaacttcctctctgcagcgtggtgtaccgtcccgtttctctggcagcggttctggtacggattttaccctgaccatctcaagcctccagcctgaagattttgccacctattattgtcagcaatcttactcttttccgtttacgttcgggcagggaactaaagtggaaattaaa

SEQ ID NO: 55 - DNA, 729 bp, synthetic construct
  source 1..729: mol_type = other DNA
gaagtacagttggtcgaaagtggcggtggcctcgtgcaaccgggtggttcactgcgtctgagctgcgccgcctcgggttttactttctctctttatggtatgcactgggttcgtcaggcgccgggcaagggtctcgaatgggtttcatctatctacggttctggtggtcacactggttatgccgattcagtgaagggtcgctttaccatttcccgtgacaactctaagaatactctgtatctgcagatgaactcgctgcgtgccgaagacacggccgtctattattgcgccaaacagcatgcataccgttactcttacgcattcgatgtttggggtcagggcactttagtgaccgtctcatcgggtggaggcggttcaggcggaggtggatccggcggtggcggatcggacattcaaatgacgcagagtccctcctcactgagtgctagcgtgggcgatcgtgtgacaattacttgtcgcgctagccagtctatctctaattggctgaactggtatcagcagaaaccgggcaaggcgccaaaattgctgatttacgcaacttcctctctgcagcgtggtgtaccgtcccgtttctctggcagcggttctggtacggattttaccctgaccatctcaagcctccagcctgaagattttgccacctattattgtcagcaatcttactcttttccgtttacgttcgggcagggaactaaagtggaaattaaa

SEQ ID NO: 56 - DNA, 135 bp, synthetic construct
  source 1..135: mol_type = other DNA
accacgacgccagcgccgcgaccaccaacaccggcgcccaccatcgcgtcgcagcccctgtccctgcgcccagaggcgtgccggccagcggcggggggcgcagtgcacacgagggggctggacttcgcctgtgat

SEQ ID NO: 57 - DNA, 72 bp, synthetic construct
  source 1..72: mol_type = other DNA
atctacatctgggcgcccttggccgggacttgtggggtccttctcctgtcactggttatcaccctttactgc

SEQ ID NO: 58 - DNA, 126 bp, synthetic construct
  source 1..126: mol_type = other DNA
aaacggggcagaaagaaactcctgtatatattcaaacaaccatttatgagaccagtacaaactactcaagaggaagatggctgtagctgccgatttccagaagaagaagaaggaggatgtgaactg

SEQ ID NO: 59 - DNA, 337 bp, synthetic construct
  source 1..337: mol_type = other DNA
agagtgaagttcagcaggagcgcagacgcccccgcgtacacagcagggccagaaccagctctataacgagctcaatctaggacgaagagaggagtacgatgttttggacaagagacgtggccgggaccctgagatggggggaaagccgagaaggaagaaccctcaggaaggcctgtacaatgaactgcagaaagataagatggcggaggcctacagtgagattgggatgaaaggcgagcgccggaggggcaaggggcacgatggcctttaccagggtctcagtacagccaccaaggacacctacgacgcccttcacatgcaggccctgccccctcgc

SEQ ID NO: 60 - protein, 622 aa, synthetic construct
MALPTARPLLGSCGTPALGSLLFLLFSLGWVQPSRTLAGETGQEAAPLDGVLANPPNISSLSPRQLLGFPCAEVSGLSTERVRELAVALAQKNVKLSTEQLRCLAHRLSEPPEDLDALPLDLLLFLNPDAFSGPQACTRFFSRITKANVDLLPRGAPERQRLLPAALACWGVRGSLLSEADVRALGGLACDLPGRFVAESAEVLLPRLVSCPGPLDQDQQEAARAALQGGGPPYGPPSTWSVSTMDALRGLLPVLGQPIIRSIPQGIVAAWRQRSSRDPSWRQPERTILRPRFRREVEKTACPSGKKAREIDESLIFYKKWELEACVDAALLATQMDRVNAIPFTYEQLDVLKHKLDELYPQGYPESVIQHLGYLFLKMSPEDIRKWNVTSLETLKALLEVNKGHEMSPQVATLIDRFVKGRGQLDKDTLDTLTAFYPGYLCSLSPEELSSVPPSSIWAVRPQDLDTCDPRQLDVLYPKARLAFQNMNGSEYFVKIQSFLGGAPTEDLKALSQQNVSMDLATFMKLRTDAVLPLTVAEVQKLLGPHVEGLKAEERHRPVRDWILRQRQDDLDTLGLGLQGGIPNGYLVLDLSMQEALSGTPCLLGPGPVLTVLALLLASTLA